European Patent Application EP 4 810 614 A1, published September 23, 2026. Title: 合成细胞器辅助的基因表达方法、DNA构建体和表达系统及其应用. Applicant: 小熊猫有限公司. The sequence listing filed with the application follows.

SEQUENCE LISTING (8 sequences)

SEQ ID NO: 1 - protein, 232 aa, synthetic construct
MSKGEELFTGVVPILVELDGDVNGHKFSVRGEGEGDATNGKLTLKFICTTGKLPVPWPTLVTTLTYGVQCFSRYPDHMKRHDFFKSAMPEGYVQERTISFKDDGTYKTRAEVKFEGDTLVNRIELKGIDFKEDGNILGHKLEYNFNSHNVYITADKQKNGIKANFKIRHNVEDGSVQLADHYQQNTPIGDGPVLLPDNHYLSTQSVLSKDPNEKRDHMVLLEFVTAAGITHG

SEQ ID NO: 2 - RNA, 816 nt, synthetic construct
  source 1..816: mol_type = other RNA
cagcagcagcagcagcagcagcagcagcagcagcagcagcagcagcagcagcagcagcagcagcagcagcagcagcagcagcagcagcagcagcagcagcagcagcagcagcagcagcagcagcagcagcagcagcagcagagacggagctcgtcgacgcggccgcaagcttggtaccgagctcggatcctaaggtacctaattgcctagaaaacatgaggatcacccatgtctgcaggtcgactctagaaaacatgaggatcacccatgtctgcagtattcccgggttcattagatcctaaggtacctaattgcctagaaaacatgaggatcacccatgtctgcaggtcgactctagaaaacatgaggatcacccatgtctgcagtattcccgggttcattagatcctaaggtacctaattgcctagaaaacatgaggatcacccatgtctgcaggtcgactctagaaaacatgaggatcacccatgtctgcagtattcccgggttcattagatcctaaggtacctaattgcctagaaaacatgaggatcacccatgtctgcaggtcgactctagaaaacatgaggatcacccatgtctgcagtattcccgggttcattagatcctaaggtacctaattgcctagaaaacatgaggatcacccatgtctgcaggtcgactctagaaaacatgaggatcacccatgtctgcagtattcccgggttcattagatcctaaggtacctaattgcctagaaaacatgaggatcacccatgtctgcaggtcgactctagaaaacatgaggatcacccatgt

SEQ ID NO: 3 - protein, 258 aa, synthetic construct
MASNFTQFVLVDNGGTGDVTVAPSNFANGVAEWISSNSRSQAYKVTCSVRQSSAQNRKYTIKVEVPKVATQTVGGVELPVAAWRSYLNMELTIPIFATNSDCELIVKAMQGLLKDGNPIPSAIAANSGIYANFTQFVLVDNGGTGDVTVAPSNFANGVAEWISSNSRSQAYKVTCSVRQSSAQNRKYTIKVEVPKVATQTVGGVELPVAAWRSYLNMELTIPIFATNSDCELIVKAMQGLLKDGNPIPSAIAANSGIY

SEQ ID NO: 4 - protein, 254 aa, synthetic construct
MELHFNLELVETYKSNSQKARILTEDWVYRQSYCPNCGNNPLNHFENNRPVADFYCNHCSEEFELKSKKGNFSSTINDGAYATMMKRVQADNNPNFFFLTYTKNFEVNNFLVLPKQFVTPKSIIQRKPLAPTARRAGWIGCNIDLSQVPSKGRIFLVQDGQVRDPEKVTKEFKQGLFLRKSSLSSRGWTIEILNCIDKIEGSEFTLEDMYRFESDLKNIFVKNNHIKEKIRQQLQILRDKEIIEFKGRGKYRKL

SEQ ID NO: 5 - protein, 5 aa, synthetic construct
GSHHW

SEQ ID NO: 6 - protein, 544 aa, synthetic construct
MGKKAEYGQGHPIFLEYAEQIIQHKEYQGMPDLRYPDGRIQWEAPSNRKSGIFKDTNIKRRKWWEQKAISIGIDPSSNQWISKTAKLIHPTMRKPCKKCGRIMDLRYSYPTKNLIKRIRKLPYVDESFEIDSLEHILKLIKRLVLQYGDKVYDDLPKLLTCKAVKNIPRLGNDLDTWLNWIDSVYIPSEPSMLSPGAMANPPDRLDGFHSLNECCRSHADRGRWEKNLRSYTTDRRAFEYWVDGDWVAADKLMGLIRTNEQIKKETCLNDNHPGPCSADHIGPISLGFVHRPEFQLLCNSCNSAKNNRMTFSDVQHLINAENNGEEVASWYCKHIWDLRKHDVKNNENALRLSKILRDNRHTAMFILSELLKDNHYLFLSTFLGLQYAERSVSFSNIKIENHIITGQISEQPRDTKYTEEQKARRMRIGFEALKSYIEKENRNALLVINDKIIDKINEIKNILQDIPDEYKLLNEKISEQFNSEEVSDELLRDLVTHLPTKESEPANFKLARKYLQEIMEIVGDELSKMWEDERYVRQTFADLD

SEQ ID NO: 7 - protein, 86 aa, synthetic construct
FVNQHLCGSHLVEALYLVCGERGFFYTPKTRREAEDLQVGQVELGGGPGAGSLQPLALEGSLQKRGIVEQCCTSICSLYQLENYCN

SEQ ID NO: 8 - protein, 243 aa, synthetic construct
AELEHLAQNISKSHLETCQYLREELQQITWQTFLQEEIENYQNKQREVMWQLCAIKITEAIQYVVEFAKRIDGFMELCQNDQIVLLKAGSLEVVFIRMCRAFDSQNNTVYFDGKYASPDVFKSLGCEDFISFVFEFGKSLCSMHLTEDEIALFSAFVLMSADRSWLQEKVKIEKLQQKIQLALQHVLQKNHREDGILTKLICKVSTLRALCGRHTEKLMAFKAIYPDIVRLHFPPLYKELFTS